European Patent Specification EP 3 438 245 B1, published January 11, 2023. Title: Coryneform transformant and method of producing protocatechuic acid or its salts using thereof. Applicant: Research Institute of Innovative Technology for the Earth SUMITOMO BAKELITE CO.,LTD. The sequence listing filed with the application follows.

SEQUENCE LISTING (162 sequences)

SEQ ID NO: 1 - DNA, 3341 bp, Corynebacterium glutamicum
atgacgctgtcacctgaacttcaggcgctcactgtacgcaattacccctctgattggtccgatgtggacaccaaggctgtagacactgttcgtgtcctcgctgcagacgctgtagaaaactgtggctccggccacccaggcaccgcaatgagcctggctccccttgcatacaccttgtaccagcgggttatgaacgtagatccacaggacaccaactgggcaggccgtgaccgcttcgttctttcttgtggccactcctctttgacccagtacatccagctttacttgggtggattcggccttgagatggatgacctgaaggctctgcgcacctgggattccttgaccccaggacaccctgagtaccgccacaccaagggcgttgagatcaccactggccctcttggccagggtcttgcatctgcagttggtatggccatggctgctcgtcgtgagcgtggcctattcgacccaaccgctgctgagggcgaatccccattcgaccaccacatctacgtcattgcttctgatggtgacctgcaggaaggtgtcacctctgaggcatcctccatcgctggcacccagcagctgggcaacatcatcgtgttctgggatgacaaccgcatctccatcgaagacaacactgagatcgctttcaacgaggacgttgttgctcgttacaaggcttacggctggcagaccattgaggttgaggctggcgaggacgttgcagcaatcgaagctgcagtggctgaggctaagaaggacaccaagcgacctaccttcatccgcgttcgcaccatcatcggcttcccagctccaaccatgatgaacaccggtgctgtgcacggtgctgctcttggcgcagctgaggttgcagcaaccaagactgagcttggattcgatcctgaggctcacttcgcgatcgacgacgaggtcatcgctcacacccgctccctcgcagagcgcgctgcagagaagaaggctgcatggcaggtcaagttcgatgagtgggcagctgccaaccctgagaacaaggctctgttcgatcgcctgaactcccgtgagcttccagcgggctacgctgacgagctcccaacatgggatgcagatgagaagggcgtcgcaactcgtaaggcgtccgaggctgcacttcaggcactgggcaagacccttcctgagctgtggggcggttccgctgacctcgcaggttccaacaacaccgtgatcaagggctccccttccttcggccctgagtccatctccaccgagacctggtctgctgagccttacggccgtaacctgcacttcggtatccgtgagcacgctatgggatccatcctcaacggcatttccctccacggtggcacccgcccatacggcggaaccttcctcatcttctccgactacatgcgtcctgcagttcgtcttgcagctctcatggagaccgacgcttactacgtctggacccacgactccatcggtctgggcgaagatggcccaacccaccagcctgttgaaaccttggctgcactgcgcgccatcccaggtctgtccgtcctgcgtcctgcagatgcgaatgagaccgcccaggcttgggctgcagcacttgagtacaatgaaggccctaagggtcttgcactgacccgccagaacgttcctgttctggaaggcaccaaggagaaggctgctgaaggcgttcgccgcggtggctacgtcctggttgagggttccaaggaaaccccagatgtgatcctcatgggctccggctccgaggttcagcttgcagttaacgctgcgaaggctctggaagctgagggcgttgcagctcgcgttgtttccgttccttgcatggattggttccaggagcaggacgcagagtacatcgagtccgttctgcctgcagctgtgaccgctcgtgtgtctgttgaagctggcatcgcaatgccttggtaccgcttcttgggcacccagggccgtgctgtctcccttgagcacttcggtgcttctgcggattaccagaccctgtttgagaagttcggcatcaccaccgatgcagtcgtggcagcggccaaggactccattaacggttaattgccctgctgtttttagcttcaacccggggcaatatgatcctccggaattttattgccccgggttgttgttaatcggtataaagggtcttaagcacatcccttacttgcctgctctccttgagcgcagttcaagaacaattcttttaaggaaaatttagtttcatgtctcacattgatgatctggcacagctcggcacttccacttggctcgacgacctctcccgcgagcgcattacttccggcaatctcagccaggttattgaggaaaagtctgtagtcggtgtcaccaccaacccagctattttcgcagcagcaatgtccaagggcgattcctacgacgctcagatcgcagagctcaaggccgctggcgcatctgttgaccaggctgtttacgccatgagcatcgacgacgttcgcaatgcttgtgatctgtttaccggcatcttcgagtcctccaacggctacgacggccgcgtgtccatcgaggttgacccacgtatctctgcggaccgcgacgcaaccctggctcaggccaaggagctgtgggcaaaggttgatcgtccaaacgtcatgatcaagatccctgctaccccaggttctttgccagcaatcaccgacgctttggctgagggcatcagtgttaacgtcaccttgatcttctccgttgctcgctaccgcgaagtcatcgctgcgttcatcgagggcatcaagcaggcagctgcaaacggccacgacgtatccaagatccactctgtggcttccttcttcgtctcccgcgtcgacgttgagatcgacaagcgcctcgaggcaatcggatccgatgaggctttggctctgcgtggcaaggcaggcgttgccaacgctcagcgcgcttacgctgtgtacaaggagcttttcgacgccgccgagctgcctgaaggcgccaacactcagcgcccactgtgggcatccaccggcgtgaagaaccctgcgtacgctgcaactctttacgtttccgagctggctggtccaaacaccgtcaacaccatgccagaaggcaccatcgacgctgttctggaactgggcaacctgcacggtgacaccctgtccaactccgcggcagaagctgacgctgtgttctcccagcttgaggctctgggcgttgacttggcagatgtcttccaggtcctggagaccgagggcgtggacaagttcgttgcttcttggagcgaactgcttgagtccatggaagctcgcctgaagtag

SEQ ID NO: 2 - DNA, 1053 bp, Escherichia coli
atgaattatcagaacgacgatttacgcatcaaagaaatcaaagagttacttcctcctgtcgcattgctggaaaaattccccgctactgaaaatgccgcgaatacggttgcccatgcccgaaaagcgatccataagatcctgaaaggtaatgatgatcgcctgttggttgtgattggcccatgctcaattcatgatcctgtcgcggcaaaagagtatgccactcgcttgctggcgctgcgtgaagagctgaaagatgagctggaaatcgtaatgcgcgtctattttgaaaagccgcgtaccacggtgggctggaaagggctgattaacgatccgcatatggataatagcttccagatcaacgacggtctgcgtatagcccgtaaattgctgcttgatattaacgacagcggtctgccagcggcaggtgagtttctcgatatgatcaccccacaatatctcgctgacctgatgagctggggcgcaattggcgcacgtaccaccgaatcgcaggtgcaccgcgaactggcatcagggcttttttgtccggtcggcttcaaaaatggcaccgacggtacgattaaagtggctatcgatgccattaatgccgccggtgcgccgcactgcttcctgtccgtaacgaaatgggggcattcggcgattgtgaataccagcggtaacggcgattgccatatcattctgcgcggcggtaaagagcctaactacagcgcgaagcacgttgctgaagtgaaagaagggctgaacaaagcaggcctgccagcacaggtgatgatcgatttcagccatgctaactcgtccaaacaattcaaaaagcagatggatgtttgtgctgacgtttgccagcagattgccggtggcgaaaaggccattattggcgtgatggtggaaagccatctggtggaaggcaatcagagcctcgagagcggggagccgctggcctacggtaagagcatcaccgatgcctgcatcggctgggaagataccgatgctctgttacgtcaactggcgaatgcagtaaaagcgcgtcgcgggtaa

SEQ ID NO: 3 - DNA, 2964 bp, Corynebacterium glutamicum
atgctaggcatgcttcgatggactacagcaggtgaatcccacggccaggcgcttatcgccacggttgaacacatgccagcaggcgtgcccgtgactaaagatgaggtctcgtatcaattggcgcgccgacgccttggatatggtcgcggcgctcgcatgaagtttgagcaagacgcgttgaccttcctgaccggcatccgccacggcctcactttgggtagccccatctcaatcatgatcggcaacactgagtgggataagtggaccaccatcatgtcctctgacgctttggacatggaagacccagacaacgttgcggcgatgtcttcgggtcgcggtgcaaaactgactcgtccgcgtccaggccacgcagattacgcaggcatgctcaagtacggattcgatgatgcccgcaacgtgctggagcgttcttcagcccgtgagacggcagctcgcgtggcagcagcaaccgttgcgcgttccttcctccgtgaaaccttgggcgtggaggtgctctctcacgtaatttccattggtgcgtccgagccttacgtcggcgcggagccaacctttgcagatattcaagcaatcgatgattccccagttcgtgcattcggtaaagacgctgaaaaatccatgatcgcggaaatcgaggccgcaaagaaagccggcgataccctcggtggcatcgtggaagtgattgttgaaggcctacccatcggtttgggctcacacatttctggcgaagatcgcctcgatgcgcagatcgcagctgcactcatgggcattcaggccatcaagggcgtggaaatcggtgacggtttcgaagaagctcgtcgacgtggctccgaagcccacgatgaagtgttcctggatgacaacggcgtataccgcaacaccaaccgtgcaggtggcctcgaaggcggcatgaccaacggtgaaaccctgcgcgttcgtgctggcatgaagccaatttctactgtgcctcgcgccctgaaaaccattgatatggaaaacggcaaggcagcaaccggaatccaccagcgttccgacgtgtgcgctgttccagccgccggtgtcgttgcagaagcaatggtcaccctggttctcgcccgcgcagtcctgcagaaattcggcggtgactccctgagtgaaaccaagagcaacattgacacctacctcaaaaacattgaggaacgaatgaaattcgaaggtttagaggatggagcgtaatgaagtgaatgatcaaattcacttagatcatcaatcagatgacacctctgaatgctcctgcccgatcgtggttcttgtgggtttgccaggagctggaaaatccaccattggacgtcgattagcgcgcgccttaaacactgaactcgtcgactccgacgaactcattgagcgcgccaccggaaaagcctgcggcgccgtgttcagcgagctcggcgagccagccttccgcgagctcgaggccatccacgtggccgaagcactgaaatcctccggagtggtgagcttgggaggcggatctgtgctgacagaatccacccgtgaactgctcaaaggccacgacgtggtctggatcgacgtgccagtagaagaaggcatcaggcgcaccgcaaacgagcgttcccgccccgtgctgcaagccgccgaccccgccgagcactaccgcaacctggtgaaagtgcgcaccccgttgtacgaagaggtggcaacctaccgacttcgcaccaacaaccgcagcccccagcaagtggtggcagcagtgttgcatcatctagaaatcgattaattaaaccgggcacctgattaacattgggctgcccggtttcttcctattacaagcgaaaggcaacgtgccccatgagcgcagcgcagattttcaacaccgtccacgtcaatggatcttccccctatgatgtccacattggttccggcctcaacgagctcattgttcagcgcgcagcggaatcaggcgcggagcaggtagcgattttgcaccagcccagcatggatgacattgcatccgagttggatgcagcactagtcgctgctggtttgaaggtcctgcaccttaatgttcccgatgcggaaaacggcaagtccttggaagtagcggggcagtgctgggatgaattgggtggcgcagcattcggccgccgcgatatcgtcatcggacttggtggcggtgctgccacagatctcgcgggattcgtcgctgctgcgtggatgcgtggcgtgcgcgtcattcaggttccaaccaccttgttggccatggtggacgctgcggtgggcggcaagactggcatcaataccgccgcaggcaagaaccttgtgggcgcgttccacgagcctgacgcagtattcattgacaccgaacgcctagccaccctgcctgacgcggaaatcatcgcgggatccgccgaaatcatcaaaactggtttcatcgccgacccagaaatcctgcgcctttacgaaactgatcccgcagcctgcctgaagaaagaagtcgaaggctcccacctacctgaactgatttggcgctccgtcaccgtcaagggctccgtggtcggccaagacctcaaagaatctagcctgcgcgaaatcctcaactacggacacacctttgcccacgccgtcgaactccgcgaaaacttccgctggcgccacggcaatgccgttgcagtgggcatgatgttcatcgctaacctctcccacaagctcgggcttatcgacgcgcccctcctcgagcgccaccgctcaatcctggcggccatcggtctgcccacttcctacgaaggcggagccttcgacgagctttacgacggcatgacccgcgacaagaaaaaccgcgacggcaacatccgcttcgtcgcactgaccgccgtgggcgaggttacccgcattgaggggccctcaaaacaagatttacagagtgcttatgaggcaatcagccactaa

SEQ ID NO: 4 - DNA, 1293 bp, Corynebacterium glutamicum
atggtctttgtgtctgattcgtctatctctttgcccatttgggatgctccgcgcgctcgcggccccatagtctcggacctggctatccctggttccaagtcgatcaccaaccgcgccctcatcttggctgcgctcgcatcaactccatccaccatcattgatgtccttcgtagtcgtgataccgatctcatgactgatggtctacgcagcctcggaatcaccattactgaagaggcagtcgatcgctaccgcgttgagcccggacagttgtctgctggctccgttgagtgtggtcttgctggtacggtcatgcgctttttgcctcctgttgctgctttcgctgatggtcctgttcattttgatggcgatcctcaagctcgtgttcgtccgatgaccagcattttggatgcgctgcgttcgcttggtgtggaggtggacaacaacaatctgcctttcactgttaatgctggtgaggtccctgagggtggcgtggttgagattgatgcttccggctcatctcagtttgtttctggtcttttgctttcagcgcctcgttttaaaaatggcgtcaccgttaagcacgtcggtggtcgtctgccgagcatgccgcatattgagatgaccgtcgatatgcttcgttccgcaggcattgagatcgaagagtcagaaaatcagtgggttgttcatcctggtgagatcttgggtcggacctggcgcattgagccggatctttctaatgcgactccgttcctagctgccgctgcggtcactggtggaaccatcaagattaatcactggccaatcaaaactactcagcctggcgatgctattcgttcgattcttgagcgcatgggctgcgaagttgagctggttgctcagggtgaaggttacgatctgtcggtgactggtccggttgctctcaagggcattgagatcgatatgtccgatatcggtgagttgacccctaccgtggcggcgttggctgcgttggcgtcgacagagtctcgtttgaccggtattgctcatcttcgtggccatgagacggatcgtttggctgcgttgactgcggagatcaacaaacttggtggaaagtgcactgagcttaaggatggtctgttgattgagcctgcgtcgctgcacggtggtgtgtggcattcatatgctgatcatcgtatggctactgctggtgcgatcattggcctcgcggttgatgacgttcaggttgaagacattaagaccacttccaagactttccctggttttgaaaatgtttgggaggagatggttggctag

SEQ ID NO: 5 - DNA, 438 bp, Corynebacterium glutamicum
atgcttggaaaaattctcctcctcaacggcccaaacctgaacatgctgggcaaacgcgagcctgacatttacggacacgacaccttggaagacgtcgtcgcgctggcaaccgctgaggctgcgaagcacggccttgaggttgaggcgctgcagagcaatcacgaaggtgagctaatcgatgcgctgcacaacgctcgcggcacccacatcggttgcgtgattaaccccggcggcctgactcacacttcggtggcgcttttggatgcggtgaaggcgtctgagcttcctaccgttgaggtgcacatttccaatccgcatgcccgtgaagagttccgccaccattcttacatttccctcgccgcggtctccgttatcgctggcgctggcatccagggttaccgtttcgcggtcgatatcctggcaaatctcaaaaagtag

SEQ ID NO: 6 - DNA, 831 bp, Corynebacterium glutamicum
atgggttctcacatcactcaccgggcggccgtactcggctcacccatcgagcattccaaatccccagtcctccacaacaccggctataaagccctcggactggaccaatgggaatacgaccgctttgagtgcaccggcgacatgctccccggaatcgtctccggcgctgatgaaacctaccgcggattctccgtcactatgccgtccaaattcgcagccctcgaattcgccgacgaagtaaccgaacgcgcccgcgccatcggctccgcaaacacacttctgcgcaccgaaaccggatggcgcgcagacaacaccgacgtcgacggcatcaggggagccctcggtgaactcctcggcagcgcatcactggccggcaaacacgccatcgtcatcggctccggcggcaccgcacgccccgccatctgggcactcatcgaagccggggtcgcgcggatcacggtgctcaaccgctccgatcgaaccgccgaactgcaaacgcttttcgacgaaacccccaccaccttggcctacgccccgctcgaacatctcgacatcgaagccgacgtcgtagtctctacagtgccctccgcagcaatcgcaggcctcgaagacacactcgcaatcgccccagtcctcgacgtcatctacgatccttggccaacaccactcgtagaagtcgcacgagccaaaggtctcaaagctgtcggaggccacgtcatgctggcacaccagtcctacggacagtttgaacaattcaccggaatggatgcaccccgcgatgctatgcgtgaggctttggaagaatccctaggcatctcggaagaacactag

SEQ ID NO: 7 - DNA, 1857 bp, Corynebacterium glutamicum
atgcgtacatccattgccactgtttgtttgtccggaactcttgctgaaaagctgcgcgcagctgcagatgctggatttgatggtgtggaaatcttcgagcaggacttggtggtttccccgcattcggcagagcagattcgtcagcgggctcaggatttgggattaaccctggatctgttccagccgtttcgagatttcgaaggtgtggaagaagagcagtttctgaagaatctgcaccgcttggaagagaagttcaagctgatgaacaggcttggcattgagatgatcttgttgtgttccaatgtgggcaccgcgaccatcaatgatgatgaccttttcgtggagcagttgcatcgtgcagcagatttggctgagaagtacaacgtcaagattgcttatgaagcgttggcgtggggcaagtttgtcaatgattttgagcatgcgcatgcacttgtggagaaggtgaatcacaaggcgctgggaacctgcttggatacgttccatattctttcccgtggttgggaaaccgacgaggtggaaaacatcccggcggagaagatcttctttgttcagttggcggatgcaccgaagctgagcatggacattttgtcctggtcgcgtcaccaccgtgttttccctggtgaaggcgatttcgatctggtgaaattcatggttcatctggccaagacgggttatgatggcccgatttctttggagatcttcaacgattccttccgcaaggccgaggttggtcgcaccgcgattgatgggttgcgttctttgcgttggttggaagatcagacctggcatgcgctaaatgctgaggatcgtccaagcgcactagagctgcgtgcacttcctgaggtcgcggaacctgaaggcgttgatttcattgagatcgccactggacgtttgggtgagaccattcgggttcttcatcaattgggtttccgcttgggtggtcatcactgcagtaagcaggattaccaggtatggacccagggcgatgtgcgcattgtggtgtgtgatcgtggggccaccggggctccaaccacgatctctgcgatgggctttgacacccctgatccagaagccgcgcatgcccgtgcggaattgctgcgggctcagacaattgatcgtccccacatcgagggtgaagttgaccttaaaggtgtgtacgcgccggatggggtggagctgtttttcgcggggccgagccccgatggaatgcccgagtggctgccggaattcggcgtcgaaaagcaagaagctggtctcattgaagccatcgaccacgtcaatttcgcccagccatggcaacattttgatgaggcagtgctgttttacaccgcgctgatggcgttagagactgtgcgtgaggatgagttcccgagcccaattggtttggtgcgcaatcaggtgatgcgttcgccgaatgatgcggtgcggttgctgctcagcgtggcgccggaggacggtgagcagggagatttcctcaacgcggcctacccggagcacattgcgttggccacggcggacatcgtggcggtggctgaacgtgcgcgcaaacgaggcctggatttcttgcccgtcccagagaattactacgacgatgtgcaggcgcgttttgatttgccgcaggaattcttggacacactcaaggaaaaccacctgctttacgactgcgacgagaacggcgaattcctccacttttacacccgcacgttgggcacgctgttcttcgaagtggtggaacgccgcggcggttttgcaggttggggcgaaacaaacgctccggtgcggttagcggcgcagtatcgtgaggtgcgggacctcgagcggggaatccccaactag

SEQ ID NO: 8 - DNA, 1188 bp, Corynebacterium glutamicum
atgaaccacgtaccagtggcaattattggcgcaggaccagcaggactgaccctcgcccacctcctccaccttcaaggtgtggaatcaatcgtctttgaatcccgcacccgcaaggacgtcgaagaaaccgtccgagcaggcattctggaacaaggcaccctgaatctgatgcgcgaaaccggagtcggcgcacgcatggaagcagaagccgatcacgatgaagcaatcgacatctccatcaacaatgagcgcacccgcattccgctgaccgaactcaccggccacaaggttgcgatctacccgcagcacgaatacctcaaagatttcattgccaagcgcatcgaagacggcggcgaactccttttcaccaccactgttgattccgtagagaactacgaaggcgacctcgccaaggtgacctacaccgaagccgatggttcctccaccaccatcaccgccgactacgtcatcgcagctgacggctccaactccccttaccgcaagttgatcaccgaagacggcggcgtgcgcgcccgccatgaatacccttacgcatggttcggcattttggtcgaagcaccaaaaacccaaaaggaactcatctacgcaacccaccctgagggctttgcgctgatctccacccgcaccgatgaaatccagcgctactacctgcagtgcaacccagacgacaccccagacatgtggtccgatgaccgcatttgggaacagctgcatctgcgtgcggactcccctggcatcaccgtgtctgaagggcgcatctttgacaaggccgtgctgcgtttccgctccgcggtcaccgaaccaatgcaaaagggacgcctcttccttgctggcgatgctgcacacaccgtgccgccaaccggagctaagggcctcaacttggctgttgccgatgtcgcagtactcgcgccagcactggttcgtgccctgaagaagaaggacaccggcttgctcgatagctacacctccctggcagtcccccgcatctggaaagcacagcacttctcctactggatgagctccatgctccacgcagtacccggcgaagatcactttgccacccagcgccgattcgctgaattgcgctccgtcctagaatcccaatccggccaacgctacctcgcagagcagtacgttgggcgcgacctaccacgcttcgaggtataa

SEQ ID NO: 9 - DNA, 504 bp, Providencia rustigianii
atgcatgaaacaatttttacccatcatcccattgattggctaaacgaggatgatgagtcagttcctaacagtgtactagattggctgcaagagcgtggttcaatgactaaacggttcgagcagcattgccaaaaagtcacggtaattccctatttagagcgctatatcactccagagatgctgagcgctgatgaagccgagcgtttacccgaaagtcaacgttactggttgcgagaagtcattatgtatggggataatattccgtggttgataggcagaacattgatccctgaagagaccctcaccaacgatgataaaaagctggtggacattggtcgtgtgccattagggcgttacctttttagtcatgatagtcttacccgagattatattgatattggcaccagtgcggatcgttgggtgcgacgttctctgctgagattatctcaaaagcccttattattaactgaaatatttttacctgaatcacctgcatatagataa

SEQ ID NO: 10 - DNA, 26 bp, Artificial sequence
  PCR primer
ctctcatatgacgctgtcacctgaac

SEQ ID NO: 11 - DNA, 28 bp, Artificial sequence
  PCR primer
ctctcatatgctacttcaggcgagcttc

SEQ ID NO: 12 - DNA, 37 bp, Artificial sequence
  PCR primer
ctctgatatcatgaattatcagaacgacgatttacgc

SEQ ID NO: 13 - DNA, 30 bp, Artificial sequence
  PCR primer
ctctgatatcgacttatcaggcctgtggtg

SEQ ID NO: 14 - DNA, 24 bp, Artificial sequence
  PCR primer
tttgtccggtcggcttcaaaaatg

SEQ ID NO: 15 - DNA, 19 bp, Artificial sequence
  PCR primer
aaagccctgatgccagttc

SEQ ID NO: 16 - DNA, 31 bp, Artificial sequence
  PCR primer
ctctcatatgttacgctccatcctctaaacc

SEQ ID NO: 17 - DNA, 33 bp, Artificial sequence
  PCR primer
ctctcatatgttagtggctgattgcctcataag

SEQ ID NO: 18 - DNA, 29 bp, Artificial sequence
  PCR primer
ctctccatggtctttgtgtctgattcgtc

SEQ ID NO: 19 - DNA, 28 bp, Artificial sequence
  PCR primer
ctctccatggctagccaaccatctcctc

SEQ ID NO: 20 - DNA, 31 bp, Artificial sequence
  PCR primer
ctctcatatgcttggaaaaattctcctcctc

SEQ ID NO: 21 - DNA, 37 bp, Artificial sequence
  PCR primer
ctctcatatgctactttttgagatttgccaggatatc

SEQ ID NO: 22 - DNA, 28 bp, Artificial sequence
  PCR primer
ctctcatatgggttctcacatcactcac

SEQ ID NO: 23 - DNA, 30 bp, Artificial sequence
  PCR primer
ctctcatatgctagtgttcttccgagatgc

SEQ ID NO: 24 - DNA, 30 bp, Artificial sequence
  PCR primer
ctttgaccatatgcgtacatccattgccac

SEQ ID NO: 25 - DNA, 34 bp, Artificial sequence
  PCR primer
ctagttccatatgctagttggggattccccgctc

SEQ ID NO: 26 - DNA, 26 bp, Artificial sequence
  PCR primer
ctctcatatgaaccacgtaccagtgg

SEQ ID NO: 27 - DNA, 31 bp, Artificial sequence
  PCR primer
ctctcatatgttatacctcgaagcgtggtag

SEQ ID NO: 28 - DNA, 36 bp, Artificial sequence
  PCR primer
ctctcatatgcatgaaacaatttttacccatcatcc

SEQ ID NO: 29 - DNA, 42 bp, Artificial sequence
  PCR primer
ctctcatatggattatgttagatagttatctatatgcaggtg

SEQ ID NO: 30 - DNA, 30 bp, Artificial sequence
  PCR primer
ctctgtcgaccttattcgtcgtagtgccag

SEQ ID NO: 31 - DNA, 30 bp, Artificial sequence
  PCR primer
ctctgtcgacatcatcgcggtgtcacagtt

SEQ ID NO: 32 - DNA, 26 bp, Artificial sequence
  PCR primer
ctctagatctcatgggcaactcctcg

SEQ ID NO: 33 - DNA, 29 bp, Artificial sequence
  PCR primer
ctctagatctatgcttgtcacatgaggcg

SEQ ID NO: 34 - DNA, 33 bp, Artificial sequence
  PCR primer
ctctcctgcaggctgaccaggatttatctgtcc

SEQ ID NO: 35 - DNA, 31 bp, Artificial sequence
  PCR primer
ctctcctgcagggatcgtcaccttccaaacc

SEQ ID NO: 36 - DNA, 29 bp, Artificial sequence
  PCR primer
ctctagatcttctaggccaggaactaacg

SEQ ID NO: 37 - DNA, 27 bp, Artificial sequence
  PCR primer
ctctagatctgaagggtgcttcgcttc

SEQ ID NO: 38 - DNA, 34 bp, Artificial sequence
  PCR primer
ctctcctgcagggtggatacaaatgggatgtctg

SEQ ID NO: 39 - DNA, 32 bp, Artificial sequence
  PCR primer
ctctcctgcagggatgaagttgctgaagcagg

SEQ ID NO: 40 - DNA, 28 bp, Artificial sequence
  PCR primer
ctctgtcgaccagatggcagttgaggtg

SEQ ID NO: 41 - DNA, 30 bp, Artificial sequence
  PCR primer
ctctgtcgaccgatcagtggagatcaacac

SEQ ID NO: 42 - DNA, 30 bp, Artificial sequence
  PCR primer
ctctgtcgacattcctgcgtctggtggtct

SEQ ID NO: 43 - DNA, 30 bp, Artificial sequence
  PCR primer
ctctgtcgacccgaccaatgatgtaactgc

SEQ ID NO: 44 - DNA, 33 bp, Artificial sequence
  PCR primer
ctctgtcgacctgtggtgactttattgtctagg

SEQ ID NO: 45 - DNA, 31 bp, Artificial sequence
  PCR primer
ctctgtcgacgccagcttctgtaagtaactc

SEQ ID NO: 46 - DNA, 41 bp, Artificial sequence
  PCR primer
ctctagatctgtgctgatcttaatattgaatcgttttattc

SEQ ID NO: 47 - DNA, 30 bp, Artificial sequence
  PCR primer
ctctagatctgactactgtgagtggcttga

SEQ ID NO: 48 - DNA, 30 bp, Artificial sequence
  PCR primer
ctctgcatgctcaacgagctgatggagctt

SEQ ID NO: 49 - DNA, 30 bp, Artificial sequence
  PCR primer
ctctgcatgccgtggtgtatctgtaactgc

SEQ ID NO: 50 - DNA, 30 bp, Artificial sequence
  PCR primer
ctcttctagaagacatcggagcaatcggct

SEQ ID NO: 51 - DNA, 30 bp, Artificial sequence
  PCR primer
ctcttctagagtccgcagaggaaccattca

SEQ ID NO: 52 - DNA, 30 bp, Artificial sequence
  PCR primer
ctctgagctcgtgaacatatcggcatcgag

SEQ ID NO: 53 - DNA, 30 bp, Artificial sequence
  PCR primer
ctctgtcgacctatggcgttctatactgcg

SEQ ID NO: 54 - DNA, 30 bp, Artificial sequence
  PCR primer
ctcttctagatatgcaagaagcaagcaagt

SEQ ID NO: 55 - DNA, 30 bp, Artificial sequence
  PCR primer
ctctctcgagtctcataaaagttctccgat

SEQ ID NO: 56 - DNA, 28 bp, Artificial sequence
  PCR primer
atgcatgcacgtactccgaagatgtatg

SEQ ID NO: 57 - DNA, 28 bp, Artificial sequence
  PCR primer
atgcatgcttacatgcctatgcattcgg

SEQ ID NO: 58 - DNA, 30 bp, Artificial sequence
  PCR primer
ctcttctagagatcggtagaacagcgtaac

SEQ ID NO: 59 - DNA, 30 bp, Artificial sequence
  PCR primer
ctctgagctcgccaagtcatgaaggttgtc

SEQ ID NO: 60 - DNA, 30 bp, Artificial sequence
  PCR primer
ctctagtactcaacaggagttggagatgtc

SEQ ID NO: 61 - DNA, 31 bp, Artificial sequence
  PCR primer
ctctagtactgatgatcctgatgccactatc

SEQ ID NO: 62 - DNA, 30 bp, Artificial sequence
  PCR primer
ctctcctgcaggtccagtgtggatcgcaac

SEQ ID NO: 63 - DNA, 33 bp, Artificial sequence
  PCR primer
ctctcctgcagggaggatatggtgactagcttg

SEQ ID NO: 64 - DNA, 30 bp, Artificial sequence
  PCR primer
ctctgatatccttcctaaacgatgagcgag

SEQ ID NO: 65 - DNA, 30 bp, Artificial sequence
  PCR primer
ctctgatatcttggtcagttcagtctggag

SEQ ID NO: 66 - DNA, 32 bp, Artificial sequence
  PCR primer
ctctcctgcaggtaatggtgtcgaccgacatc

SEQ ID NO: 67 - DNA, 32 bp, Artificial sequence
  PCR primer
ctctcctgcaggaagttagatgtggctccgac

SEQ ID NO: 68 - DNA, 32 bp, Artificial sequence
  PCR primer
ctctcctgcaggaattcgcaggatccaagctc

SEQ ID NO: 69 - DNA, 32 bp, Artificial sequence
  PCR primer
ctctcctgcagggaagcaggttcttagcgatg

SEQ ID NO: 70 - DNA, 31 bp, Artificial sequence
  PCR primer
ctctgtcgacgatagaagaagtaggcacctc

SEQ ID NO: 71 - DNA, 30 bp, Artificial sequence
  PCR primer
ctctgtcgaccaatctgtatggttgcctcg

SEQ ID NO: 72 - DNA, 32 bp, Artificial sequence
  PCR primer
ctctcctgcaggctcgaatgtttacctgcctg

SEQ ID NO: 73 - DNA, 32 bp, Artificial sequence
  PCR primer
ctctcctgcaggggatgtattcgatctgggac

SEQ ID NO: 74 - DNA, 30 bp, Artificial sequence
  PCR primer
ctctgtcgacctcagattggtttcgcagtc

SEQ ID NO: 75 - DNA, 40 bp, Artificial sequence
  PCR primer
ctgattgcgcaccaaaccaagaacgtatccaagcaggttc

SEQ ID NO: 76 - DNA, 20 bp, Artificial sequence
  PCR primer
ttggtttggtgcgcaatcag

SEQ ID NO: 77 - DNA, 29 bp, Artificial sequence
  PCR primer
ctctgtcgactcaacggtaggaagctcag

SEQ ID NO: 78 - DNA, 30 bp, Artificial sequence
  PCR primer
ctctgtcgacgttcttcgaagtggtggaac

SEQ ID NO: 79 - DNA, 39 bp, Artificial sequence
  PCR primer
gtgaggcagctgacatcaaacgttgaagccaaggtagag

SEQ ID NO: 80 - DNA, 20 bp, Artificial sequence
  PCR primer
tttgatgtcagctgcctcac

SEQ ID NO: 81 - DNA, 30 bp, Artificial sequence
  PCR primer
ctctgtcgactgatcaccttaaagggcgac

SEQ ID NO: 82 - DNA, 30 bp, Artificial sequence
  PCR primer
ctcttctagagaaacgatcaagtgcaccag

SEQ ID NO: 83 - DNA, 40 bp, Artificial sequence
  PCR primer
gacacgagcgtttatacctctaattgccactggtacgtgg

SEQ ID NO: 84 - DNA, 20 bp, Artificial sequence
  PCR primer
gaggtataaacgctcgtgtc

SEQ ID NO: 85 - DNA, 30 bp, Artificial sequence
  PCR primer
ctctgagctcgagaacacgaaccatacgag

SEQ ID NO: 86 - DNA, 29 bp, Artificial sequence
  PCR primer
ctcttctagatacgtcctaaacacccgac

SEQ ID NO: 87 - DNA, 40 bp, Artificial sequence
  PCR primer
gaccaaccattgctgacttgcgtatccatagtcaggcttc

SEQ ID NO: 88 - DNA, 20 bp, Artificial sequence
  PCR primer
caagtcagcaatggttggtc

SEQ ID NO: 89 - DNA, 30 bp, Artificial sequence
  PCR primer
ctcttctagatgatcagtaccaagggtgag

SEQ ID NO: 90 - DNA, 33 bp, Artificial sequence
  PCR primer
ctctcctgcagggtcattgacctggatacgatc

SEQ ID NO: 91 - DNA, 41 bp, Artificial sequence
  PCR primer
gaacacaccaaccttgaagtgcatgtcgttgtcgatgtctc

SEQ ID NO: 92 - DNA, 21 bp, Artificial sequence
  PCR primer
cacttcaaggttggtgtgttc

SEQ ID NO: 93 - DNA, 31 bp, Artificial sequence
  PCR primer
ctctcctgcagggtcatatttccgctggcac

SEQ ID NO: 94 - DNA, 32 bp, Artificial sequence
  PCR primer
ctctagtactatgcgttcttcaattgcgactg

SEQ ID NO: 95 - DNA, 30 bp, Artificial sequence
  PCR primer
ctctagtacttgaccaatgagaccaagcag

SEQ ID NO: 96 - DNA, 29 bp, Artificial sequence
  PCR primer
ctctctcatatgcgcacgtcgatcgccac

SEQ ID NO: 97 - DNA, 32 bp, Artificial sequence
  PCR primer
ctctctcatatgcgttgagcagcagaatcctg

SEQ ID NO: 98 - DNA, 32 bp, Artificial sequence
  PCR primer
ctctctcatatgaccgcttatcaggaggcaac

SEQ ID NO: 99 - DNA, 32 bp, Artificial sequence
  PCR primer
ctctctcatatgatcaacgtcttaccgcatgg

SEQ ID NO: 100 - DNA, 28 bp, Artificial sequence
  PCR primer
ctctctcatatgacgaaactccccttcc

SEQ ID NO: 101 - DNA, 31 bp, Artificial sequence
  PCR primer
ctctctcatatgcttcgtcatcacgcaggac

SEQ ID NO: 102 - DNA, 30 bp, Artificial sequence
  PCR primer
ctctctcatatgcgtctgatgcctgcgctg

SEQ ID NO: 103 - DNA, 32 bp, Artificial sequence
  PCR primer
ctctctcatatgggaagccttaccgccgaacc

SEQ ID NO: 104 - DNA, 29 bp, Artificial sequence
  PCR primer
ctctctcatatgaaactctcggtctgcac

SEQ ID NO: 105 - DNA, 33 bp, Artificial sequence
  PCR primer
ctctctcatatgggatcaaatacatgagggtcc

SEQ ID NO: 106 - DNA, 40 bp, Artificial sequence
  PCR primer
ctctcatatgaaattaacttctttacgcgtatctttattg

SEQ ID NO: 107 - DNA, 38 bp, Artificial sequence
  PCR primer
ctctcatatgttatctcattttcactgcagaacttaac

SEQ ID NO: 108 - DNA, 42 bp, Artificial sequence
  PCR primer
ggaattccatatgaatctttcagtatgcactatcacttttag

SEQ ID NO: 109 - DNA, 35 bp, Artificial sequence
  PCR primer
ggaattccatatgttaaatggcttgagcggtagtc

SEQ ID NO: 110 - DNA, 30 bp, Artificial sequence
  PCR primer
ggaattccatatgattcgcttccacctgtg

SEQ ID NO: 111 - DNA, 33 bp, Artificial sequence
  PCR primer
ggaattccatatggatgaggttcactggcagac

SEQ ID NO: 112 - DNA, 30 bp, Artificial sequence
  PCR primer
ggaattccatatgagaatcgcgctctgcac

SEQ ID NO: 113 - DNA, 33 bp, Artificial sequence
  PCR primer
ggaattccatatggtcatgtcggtctcctgaag

SEQ ID NO: 114 - DNA, 33 bp, Artificial sequence
  PCR primer
ggaattccatatgccgtcaaagctagccattag

SEQ ID NO: 115 - DNA, 35 bp, Artificial sequence
  PCR primer
ggaattccatatgttacaatgaagcagagactcgg

SEQ ID NO: 116 - DNA, 31 bp, Artificial sequence
  PCR primer
ggaattccatatgcccaaccgtctcggcatc

SEQ ID NO: 117 - DNA, 34 bp, Artificial sequence
  PCR primer
ggaattccatatgctacaaccgatgctgcacaac

SEQ ID NO: 118 - DNA, 31 bp, Artificial sequence
  PCR primer
ggaattccatatgagtgccgagaggcgactg

SEQ ID NO: 119 - DNA, 32 bp, Artificial sequence
  PCR primer
ggaattccatatggtgctgctgatcagcctgc

SEQ ID NO: 120 - DNA, 30 bp, Artificial sequence
  PCR primer
ggaattccatatgcgtacctcgatcgccac

SEQ ID NO: 121 - DNA, 33 bp, Artificial sequence
  PCR primer
ggaattccatatgcagaatccgttctgccatgg

SEQ ID NO: 122 - DNA, 30 bp, Artificial sequence
  PCR primer
ggaattccatatgggacgacaggttcgtac

SEQ ID NO: 123 - DNA, 32 bp, Artificial sequence
  PCR primer
ggaattccatatgcttcgaatcgaccgctcag

SEQ ID NO: 124 - DNA, 32 bp, Artificial sequence
  PCR primer
ggaattccatatgcctaaccgtctcggaattg

SEQ ID NO: 125 - DNA, 33 bp, Artificial sequence
  PCR primer
ggaattccatatgctaaaggcgatgctgcacag

SEQ ID NO: 126 - DNA, 43 bp, Artificial sequence
  PCR primer
ctcttcatgaaatattcgctatgtaccatttcatttcgtcatc

SEQ ID NO: 127 - DNA, 39 bp, Artificial sequence
  PCR primer
ctcttcatgactctaaacgagactctcacatcatttcac

SEQ ID NO: 128 - DNA, 507 bp, Providencia stuartii
atggatgaaacgctttttatctctcacccgataacatggctatcagaagatgatgaccttgttcctgaaaatgttttagattggctacatgaactagggtcgatgacaaaacgcttagagcagcattgccaacgtgtcacggttgttccttatacgcaacgttatgtgactcaagaggcattgagcgaagaagaagcggcgtgtttacctgtcagtgaatattattggttacgtgaagtcattatgtatggtgataatattccatggttacttggacgaacgttaattccacaggagacattgactggtgaagaccggaaacttattgatatcggtgctgtaccgttagggcgttatctctttagccatgataatctttcccgtgattatattcatatagggcagcaaaatttgcgatggatccgccgctctctattaagattatctgaaaaacctttattattaaccgaactgtttttacctgaatcacctgcatataaaagataa

SEQ ID NO: 129 - DNA, 510 bp, Cronobacter sakazakii
atgtcccatcccgcgctgagacaactgcgcgcgttgtccttttttgacgatatcagcacgcttgatagttcgctgctcgactggctgatgctggaagattccatgacccgccgtttcgaaggcttttgcgagcgcgtgacggtcgacatgctgtttgagggctttgtcggccccgaggcgctggaggaagagggcgagtttttgcctgatgagccgcgctactggctgcgcgaaatcctgctgtgcggcgacggcgtgccgtggctggttgggcgcacgctggtgccggagtctacactttgtgggccggagctggcgttgcagcagctcggtaccacgccgctgggccgttatctgtttacctcatccaccctcacgcgtgattttatccagccgggccgcagcgacgaactctggggacgccgctctctgctgaggctttccggcaaaccgctgctgctgactgaactgtttttacctgcatcacccttgtacggagaggaaaaataa

SEQ ID NO: 130 - DNA, 30 bp, Artificial sequence
  PCR primer
ctctgtcgaccagacaaccaggttgatctc

SEQ ID NO: 131 - DNA, 40 bp, Artificial sequence
  PCR primer
gatgcctagggattcttccatttggaatgctcgatgggtg

SEQ ID NO: 132 - DNA, 20 bp, Artificial sequence
  PCR primer
tggaagaatccctaggcatc

SEQ ID NO: 133 - DNA, 32 bp, Artificial sequence
  PCR primer
ctctgagctcgttactcgttaaggaagcactc

SEQ ID NO: 134 - DNA, 1863 bp, Corynebacterium casei
atgcgttcttcaattgcgactgtttgtctatcgggcactctcgcggaaaagctgcgggctgctgccgatgccggctttgacggagtagaaatctttgaacaagacttgattgtctcgccgcattcaccagaacaaattcgtgaacgtgctgcggaattgggtctcacactggacttgttccagccgttccgtgacttgctgagcgtggaagaagatatcttccgggataatctgcgccgtctggaatccaagttccagctcatgcagcgtcttggcatggaccagattttggtgtgctctaacgtggctactgccactgtggatgatgatgaagtccgcgtggatcagctgcgccgcgccggtgagttggctgcacgctatggctgcttcatctcttatgaggcattggcttggggcaagtatgttaatacttatcagcatgcttatgaccttgtggttaaggctgatcatccgaatgtgggcacgtgtttggattctttccatattctttcccgcggtgatgatccatcggggattgcggatatggatccggataaaattttcttcttgcagctcgcggacgctccgactatggagatgggaatcttaccgtggtcacgccaccaccgcgtattcccgggcgagggtgatttcgacctgaagaacttcatggagcaggtagccaaatcaggttataacggtccagtgtcgttggagattttcaatgatgaattccgcgaggctgaggtcggccggaccgcgatcgatggtctacgctcgctgatttggttggcggacaaaactgcaacacgggtgccggactcaccgttggaattaccgaagctggctgatgctcagtcaccacggggctttgactttgtggaactacgcacggggcgcctgggcgaagtcaccaaggcactgcaccaactgggattccgtttgggtggctaccaccagtccaaaccagactttcaagcgtgggtgcagggggatgttcgcatcatcgtggaggatgaaggttccaccggtggcgcaacggagctgacaggcttgggtgtcatcgtggatgatgccactgctgcggcagagcgtgccaccgcgttgaaagcaacaccagttccacgcatgaccggggaagatgaagaagacctacatccagtctttaccccagatggatctgaactgtacttttgtggaccaggacaaactggccggggaagcacatggataccggagttcggttttgaacccgatgaaaccagtagctcggagacttctgacgtattgattaattctgttcaccacattgctttggcgcagccacggcatatggctgcggaaacccgtttattttactcttcggttctgggattggaaccagctgtgccggagttcattccgtcgccagcaggtctggtgcacaagcaggcgattgaaggcgagaatgtttgcatcacagtgtcggccgctccggaaggctctgaacagggtggtttctttgctgagcactacccggaacacatcgcttttggcagtgatgacgtctttgcagttgcacaacgcgcggtgaggcgtggattgaagatgttgcccattccagagaattactatgatgacctggcagcacgcttcggactggaaccgggattcatcacgaagattaaagcactcaatatttgctatgaccgcagcagcaatggcgaatatctgcacttttacaccgcgcctttgggcaataccttctttgaggtagctgaggttcgaggggactaccgcggtttcggctgggcagatgaaccgattcgcttggccgcgcaataccgcgcgctgcgcgatgatgtccgcggaatcccgcgctaa

SEQ ID NO: 135 - DNA, 1869 bp, Corynebacterium efficiens
atgcgcacgtcgatcgccaccgtctgtttatcaggaaccctcgccgagaaactccgcgccgccgccgacgccggctttgacggcgtggaaatcttcgaacaggacctcaccgtctccccccactccccggagcagatccggcagcgggccgccgacctggggctgaccctggatctcttccagcccttccgggatttcgagggggtggaggaggaacagttcgtgaagaatctccgccgcatggaggcgaagttcgcactgatgaaccggttggggatcgacaccatcctgctgtgctccaatgtcgccaccgcgaccatcaacgatgatgaactcttcgccagccagctgcgccgcgccggggacctggcacagcgctaccaggtccgcatcgcttatgaggcgctggcgtgggggcggttcgtcaacgatttcgagcatgcccagcgcatcgtcgacatggccgaccacccccaggtgggcacctgcctggataccttccacatcctctcccgcgggtggtccaccgacgcggtggagcagatccccggcgagaagatcttcttcgtccagcttgccgatgcccccaagctcagcatggacatcctgtcctggtcccgccaccaccgggtcttccccggggagggcgatttcgacctggtgaaattcatgacccacctcgcccgcaccggatacgacggacccatctccctggagatcttcaatgattccttccgcaaggccgatgtggcccgcacggccgtcgatggtctgcggtccctgcgctggttggaggaccagacgtggcacgccctggccgaggacgaacgcgatgtgaccctgcagctgtccccgctgccggaggtcgcagaacccgccggtgtggatttcctcgagatctccaccggacggctgggggagaccatccgggtgctccaccagctgggtttccagctcggtggccaccaccgcagcaaatccgacttccaggtctggacccaggggccggtccgcatcgtcatcggtgaccgcgggcccaccggcgccgccaccaccatcaccgggctcggtttcgccaccccggatccggcctccgcgcagcagcgcgcccatctcctccaggcgggcaccatcgcccggacccgcgaggacgatgaggcagatctgcggggcgcctacgcccccgacggcaccgaggtgttcttcggtgaggtcagcccggacggattccccacctggctcgatgagttcggtgtggagaagaccgaccaggtgtccgacagcctcatcaccgggatcgaccacatcaacctcgctcagccctggcagcacttcgacgagtccatcctcttctacacctccctcatggcgctggaggcccgcgaccgcgatgagttccccagccccatcggtctgatcagcaaccaggtgatgagctcacccaatgacgccgtgcgtctgctgctcagcatcgccccggaggacggggaacagggtgatttcctggacgccgcctaccccgagcacatcgcgctcaccaccaccgatatcgtcgcggtggcccgccgtgcacgcaagcgtggcctggcgttcctccccgtcccggagaactacttcgaggacctgcaggcacgtttcgatctcgacccggagttcctggatctgctacgcgagaacaacctgctctatgaccgtgatgaccacggtggggaattcctccacttctacacccgcaccctgggcaccatgttcatcgaggtcgtggaacgccgcggtggtttcaccggctggggtgagaccaacgcaccggttcggctcgccgcccagtaccgcacgatccgcgacgccgagcgcggggtcccgcgctaa

SEQ ID NO: 136 - DNA, 1917 bp, Pantoea ananatis
atgaccgcttatcaggaggcaacaatgaaacgttctgtcgctacggtctcggtatcgggcacgctgccggaaaaactgcgagcaattgccgccgcaggcttcgatggcgttgaaattttcgataacgatctggtctattatcccggctcacccgtggaaatccgccagctgtgtgaagccctcgggctggaaatcttgctgtttcaaccttttcgcgacttcgaaggcggtccccgtgacaggctggcgcaaaacctggcgcgcgcggcgcgcaagtttgaggtcatgcaacagctgggctgtcagcggatgctggtctgcagcaatgtctcacccgactgcagtgacgacttcgccacacaggtcagcgatctcaccgctctggcagagctggcggctgagcacggtattactctcggttatgaggcgctggcctggggacgacacgtcagcctgtggcgcgacgcctgggcccgcgtcaaggccgtcaaccatcccgcgctggggatcgtgctcgacagttttcatattctgtcgcgcggcgacagcctggacgggctggaagcagtcccgacggagaaaattgtgttcgtacagctggcggatgcaccgctgctaaaaatggatgtgctgtcgtggagtcgccacttccgctgttttcccggccagggcgaattcaatctgactcagtttatgacgcaactgtcggcgcatggctaccgggatgcctggtcgctggaaattttcaacgatggattccgcgcctcgccggtggtgcctaccgcgcaggatggttatcgatcgctgctgtggctggaggagcaaacccgtgactggctggtcggacagccgctgctgccgagcgcgctggcctccctggccggggaagggctgttccactctgcgccccagccgccgctgttgtcgctggagttcattgagtttgccgtcagccacaatgacgctttggcactcggacagtggctgacgcagcttggcctggttcatgcgggcgatcatcgctccaagcaggtgtcgctgtatcgtaacggcaaggtgcatgtgattctgaatgcgcagccggagagccaggccagcgggtattatcatcagcacggtatttcgctgtgtgcggtggcctggcgggttcgcggggtcgataagctgatcacgcgcgcgcaggattacggttacgccatctggcagggggaaaccggccccaacgaacgccagatcccggcgttatgtgcgcctgacggcagcctgatttatctggtggaagatgagcctgccggtcaagacggctaccacagcgacttccacttaacgcaccgcgccgcgccccagcctgcgatgcagaccatcgaccatctggcgattgccctgccggatgatacgcgcgataactggattatgttcctgcgtagcgtgccgggttttgtgcaggataccgagtgggaactgcccgatccgctggggctggtgcgtagccgcgtgctgcgaagccccaacgatgcgattcgcctgccgctaaacatgtcggtcagtcgggaaacccagatagcccgcgctttaacgacctatcagggcgcaggtttgcagcacgtcgcctttggctgtgacgatctgttcagtgcggtaaaggccgcgcgcgaacgtgggctgaaaaccttgcacattcccgataactattatcaggacctgatggcgcgtttcgatctcgacgccgattttctggcgcagctgcagcgttacgatgtgctgtacgatcgggacgaacagggcggggagctgctgcacgtctatacgcttccctatgaaaagggccgcttcttctttgagctgctggaacgacgtggcggctatcgtggctttggcgcggccaatgctcccgtgcggctgaccgccatgcggtaa

SEQ ID NO: 137 - DNA, 852 bp, Gluconobacter oxydans
atgacgaaactccccttccctttcggcatgaacgaattcacgacccagccctggtcgttcgaggaagacgtggcgcgttaccgcgacctcggcgtggatgcgatcgagatctgtgaagccaagcttgatccggcccgcattgaggagcagatgtgcctcgtcagggagagcgggctgagcgtcagtgcggtccagccgctggtccggaccttcttcggaagcgctatggtccctgaacctgaagcgactgaagcccgcgtcaaacgccttacccaaagcctgaaaacgctcgcgcctcatgtccccggcagcgtctttgtgaccaataccggcgcgccacccaagggtaacatgcgccgtaccatggacgagacggtgcgttacctgaaggagctctgtccccttgccgaggatctgggtgtttccctgtcgctggagccgctcaacccgacctcggtgaacaccgaaagcgccatctggaccatcgagcaggccatggacatcattgaggacgtcggccatccggcgatgggtctgtgtctggattactggaacatctggcagcagaaggatgtctgcgcggctatccgtgctgcgggaagcaaaatcaacgtccttcaggtcagcgactggcgcacgccctattccgccgccgaccgcctgatccccggcgatggctgcattccgcttcatgaaatgctgcatgccacatgggatgcgggctttcgtggcgcctgcacggtcgagatcttttcgtcagatgtgccggacagcctttatgaccgcgacctgagcgatgtcatccgcttctgccgcgagggactggatcaggcctggaccggcgaggcctga

SEQ ID NO: 138 - DNA, 1473 bp, Pseudomonas putida
atgcgtctgatgcctgcgctggtggccttgctgccactgctccccctgcccgccctggccgccgcaccggccaaccccgaaaccctgcgtgtcgagcgctacgctgacgacgaccagctcggctcgctgcgctgggccatcgaaaccagtaaccagaaccccggccactacagcatcgacattgccgccgtcggccagccgccctacgtgatccgccccagccgtgcgctgccggaaatcaagggcccggtgcgcatcaccggcctgccttgggcccgcgatggccaatacatcgccatcgacggttcggcctacatcaaggaccagggcgtacgtacctgccccggcgccctgcccggccagttcggcactaacgtgcgcaccaccaccaaccccgggctggtgctgcgcgacacccagggcgtgcacctgagcggcctggaagtgcgcaacttctgcatcggcatcctggtcaaccgcgccagcggcaacgtgatcgaagacaaccgcatcgtcgccaacaaaggtggcgcgggcatcatgctgaccggtgacgacggcgcgggtaaccccaccgccaccaccacgaacaacaacaaggtgctgcgcaaccaactgatcgacaatggcgacggcctggagctgacccgcggagcggcattcaacctggtggccgacaatctgttccgctccacggcggccaaccccgaaccctcgcagggtatcgagattctgctgggcaacgacaacagcgtggtgcgcaaccgcttcgagaactactccgacggcctgcagatcaactggggcaagcgcaactacctggcggccaacaccttcagcggcaactcgatcggcgtcagcgtcaccggcgagggcaacatcctcgacggcaacctgatccacggcaaccgcatcggcgttgcactgcgcccggaaccggatgctaccgccacgcgcctgagcggcaaccgcatctggggtaacagccaggatatccgccgctgtgaagcgggcggttcgtgcgtgccgggccaacgcaccggcgccatcgtgtttggcgtgcctgcgcaggcgcatgcgctgtatgtaggttcgcgcggggtgggcgccgacttgccgaagaaagaccaggcgatcatctgcgatgccaacggcgagcccaagccttgccagccgctgcccaaccataaccagcaggcgccaaggctgattgcgctggaaggcaatgtgttgcgcggtgaagtacaggggccggaatcgagcctgctgcgggtggagttctttggcaatgccgaggcgaatggcaccgaggcggagcagtacctcggggaggtgctggtgaacagtgacagacaggggcaagcgcggtttgcacaagtgctggagaacatcggtgggttgcgcagctttaccgcgaccgtaaccactgccgatggggcaacctccgagttgagcctgccggttcggcggtaa

SEQ ID NO: 139 - DNA, 918 bp, Rhodopseudomonas palustris
atgaaactctcggtctgcaccatcacattccgccatcacctgctctgcttcagcgagatcgtcgagtggacgcaacgcaacggcttcgacggcgtcgaactgtggggcgctcatgcgcgcggcctgatgcggacgcacccggaatacgatgcagattggcttcgcagttacggcctgtcggtgccgatgctgagcgattacctgccgaccgatggcgacatcacggacactcgccaccgtgcaatcgagctctgccggattgcacagcattggtcagcgcgaaagatccgcacattcgccggtaacagaccgagcgcccagctgtcgcgcgagcagcgcagagcgctggccggccggatcggtgagatcgccggcatcgtccatgatcacggcatccggctgttggtcgagacacacccgaacacgctggccgacaacgtcgactcgacacttggcctgttggcggatgccaaccacccaggtctcggtattaacttcgatgctctgcacgtctgggaaggcggcgacgatcccgttctggctcgccgcacgctcgcggacttcatcgggcactatcatctcaagaacgtccgatcacgcgacgagctcggtgtgttcgcccctgagaacgtctattctgccgccggctcccgtgacggcatggtgccgctgtttgacggcgcgatggattacgaaggtttcctcgcatccttggcggacgagaccgatgcggaagcgtcgctcgaatggttcggtcacgattgcttcgaaaccctggcccgagatcggctagccatattcgcacgctcgatatcgacgagaggtcgccgcggctcggcgggcacgcagcaagcgcggctggcagagtcgcgtgccgccggccgcgccgcctcctccaaaggaccctcatgtatttga

SEQ ID NO: 140 - DNA, 1461 bp, Acinetobacter baylyi
atgaaattaacttctttacgcgtatctttattggcgctgggcttggtaacatcaggttttgctgcggcagaaacttatactgtagatcgttatcaggatgatagtgaaaaaggctctttgcgttgggcaattgaacaatctaatgcaaatagcgcacaagagaatcagattctgattcaggctgttggtaaggcaccttatgtgatcaaggtggataaaccgttaccaccgattaaatcatctgtaaaaattattggtacagaatgggataaaacgggcgaatttattgcgattgatggttcaaactatatcaagggcgaaggcgaaaaagcatgtccaggtgcaaatccaggacaatatggtaccaatgttcgtaccatgactttaccaggtttggttctacaagatgtcaatggtgtgaccctgaaaggtcttgatgttcatcgcttctgtattggtgtactggtaaatcgttcaagcaataatttgattcagcataaccgtatttcaaataattacggtggcgctggtgtcatgatcacgggtgatgatggtaaaggtaacccaacgtctaccaccaccaataacaacaaagtattggataatgtgtttattgacaatggcgatggtcttgaactgacgcgtggagcagcattcaacctgattgctaacaatctgtttacatcgaccaaagccaatccagagccgtctcaaggcattgaaattctttgggggaatgacaatgcagtggtgggtaacaaatttgaaaactattcagatggtctacaaatcaactggggtaaacgtaattacatcgcttataacgaattgaccaataactctttgggtttcaatcttacaggtgatggaaacatcttcgatagtaacaaagtgcatggcaatcgtattggtatcgcaattcgttctgaaaaagatgcaaatgcacgtatcacacttaccaaaaatcagatttgggataatggtaaagatatcaaacgctgtgaggctggtggttcatgtgttccaaaccaacgtttaggtgcaattgtatttggtgttcctgcgcttgagcatgaaggttttgtaggctctcgtggtggcggtgtagtcattgaacctgcaaaattacaaaaaacatgtacacagccaaatcaacaaaactgtaatgccattccgaaccaaggtattcaggcacctaaactgactgtcagtaaaaaacaacttacagttgaagttaaaggaacaccaaaccagcgttacaacgtagaattttttggaaatcgtaatgcatcttcttccgaagctgagcaatatttaggttcaattgttgtagtgacagatcatcaaggtcttgcaaaagcaaactgggcaccaaaagtcagcatgccatctgttactgcgaatgtaactgatcacttgggcgccacttcagagttaagttctgcagtgaaaatgagataa

SEQ ID NO: 141 - DNA, 846 bp, Alteromonas macleodii
atgaatctttcagtatgcactatcacttttaggcaccaacttatctcaatcgctgaaattgcaaaatggtctgtggcaaatggttttcaggggatcgaattatggggtgcacatgctacgaatttagaagaccaacccgagtatgggaaagagtggctctcaagctacgcgttgaaaacatccatgctaagcgattatctgccactttttgaagggaacgacgctttgtattttaaggttcatcgcctttgtcgtttggctaaacactggggggcaaccaagattcgcacatttgctggcaacgaaggcagcgcagccatacctgaagaccgaaaaaccctgcttttcgagcggttacaacttgtttgtgattggcttagcgactatgggcttaacttagttatcgaaacacaccctaatacttacgctgactcggtgggttctaccattgaattgtttgaaaaagttaacaaagacaatttgcaactaaattacgatgtgttgcatgtatgggaatctggcgctgacattatttcctcttgtgaacaactcgcgccatatataaatcattttcactttaaaaacataagtagcagtaaacacttaagtgtgtttgctccagacaatgtgtatgccgcagcaggctcgcgagaaggcatggtccccattttcgacggtgctgtagattatcaaaggtttattgaatacctgtactcgaaaacaactctgcgaaatattgactcttcactcgagtggtttgggaacaattgcaagaatatcctcagtcaggacagatataaattacagaaaatgagccaggccgcgactaccgctcaagccatttaa

SEQ ID NO: 142 - DNA, 876 bp, Marinobacter hydrocarbonoclasticus
atgattcgcttccacctgtgcaccatctcgttccgccaccagttggtgtcgttaccggaactcgctacctgggctggcgccaccggctttgacggtattgaactctggggcgtgcatgcctggcacctgttacagcagcccggactggatggccgctggctgcaaagccagggactggccattcccatggtcagcgactacctgccgctagacggtagcgagcaggaggctatccactacacccgcgaactctgccggctggcccgacactggcaggcccccaaactgcgaacgtttgccggccatcagggcagcgccgagctcgaccagagacagcgccaggcccagacccgacgtctgcagacgctgacccgttgcgtcgcagatgaaggcctgaccctggtggtggaaacacaccccggcaccctggccgatacggtcgactccacgctgacgttgctaaccgacgtggatcacccggccctgggtatcaacttcgacgtcttgcatgtctgggaagccggagcagacccaaagctggcgctgcaacaaatggcgccctgggtcagacattttcacttcaagaatatccgtcatcgggatcagctcggcgtatttgctccggctaatgtctactcaccggccggttcccggcagggaatggtgcctgtgctggacggtgcctgtgactaccggccgctactggacaccctggccggctggcaacagtcgcaaacccatccggccccactggacatttccctggagtggttcggcccggacagctaccgggtgctatgcagcgatcttcaccagttgcggcaaaacgttcgccagaaccacgcgcaatctcaggcgctggccgtctgccagtga

SEQ ID NO: 143 - DNA, 837 bp, Methylobacterium extorquens
atgagaatcgcgctctgcaccatcagctttcgccaccatctcgtgtcgatcggcgaactcgcccgcttcgcccgcggccacggcttcgacggcatcgaattgtggggcgtgcatgcccgcaatctcggccccggcgaccacgctgaatggctcgccgcctacggcctgcgcgtgccgatgctgagcgactacctgccgctcgacgcgccgctggaaatcctgaccgagcggacggccgaactcgcccggctcgccgggagctggggggcgccgcggctgcgcaccttcgccgggaccaagggcagtgcggccgcctcgctcgacgagcgcgcccatgtcgcccagcgcctgcggatggcggcgggccaactcgccgaccagggcctgcgcctcgtggtggagacgcatcccggcacgctcgccgacaccaccgcctcgctcctcgacctgctggatgcggtcgatcacccgaacctccgggtcaatttcgacacgctccacgtctgggaaggcggcgacgacccgctcgcggcccacgcccggctctccccgcatatcgactactatcacctcaagaacgtgcgcagccgcgccgacctgtcggtgttcgagccggccaacgtctatgccgcggccggacggcgcgagggcatgaccggcctgttcgagggcgcgctggattacgccgctttcctgaagacgctgccgccgcaggcggaaggctcgctcgaatggttcggcgaggccagcttctcggtcctgcccaccgaccttttccgcctgcgcagtgccactgccggccgccgcggggcgggagccctccacgccgcgcgctga

SEQ ID NO: 144 - DNA, 1080 bp, Neurospora crassa
atgccgtcaaagctagccattagttccatgtccctagggcgctgctttgccggccactctctggacagcaagcttgatgccgctcaacgatacggctatcttggtatcgagcttttttatgaggatctggtcgacgttgcagagcatttgtcgaacgagcgtccctctcccgaaggcccttttgtcgaagctcagatagccgccgctcgtcatattctccagatgtgtcaagccagggcgcttgaggtcgtctgcctccagcctttcatgcactacgacggccttaacgacagggcagaacatgagcgtcgtctggagaagctagcactatggattgagctcgctcatgagcttcacaccgacatcattcagatcccagccaacttcctccctgccaaccaagtcagtgacaacctcgacctgattgtctcagatctttgcaaggtggccgatattggagctcaagctttgccccctatccgctttgcctacgagagtctttgctggagcacccgtgtcgacctctgggagcgctgctgggacatcgtacaacgcgttgaccgccccaactttggcatttgccttgacaccttcaacatcctcggccgcatctatgccgaccctacatctcctagcggtaggacatccaacgcaaaagaggcagtcaggaagtccatcgccaacttggtctcgcgcgtggatgtctccaaagtcttctacgtccaggtggttgacgccgagaggctgagcaagccactactgcccggtcacccgtattacaatccagagcagccggcgaggatgagctggtcgcgcaattgtagactgttctacggcgaaacagaatatggtgcgtatcttcccgtgaaggaggttgctcgagccctttttcacggcattggtttcgagggctgggtcagtttggagcttttcaaccgcagaatgtctgaggagggacctgaagtgccggaggaacttgccatgagaggcgctatctcgtgggccaagttggtgcaagacctgaggataccggtggaggggccattggtgacgatgccccgagtctctgcttcattgtaa

SEQ ID NO: 145 - DNA, 1116 bp, Aspergillus niger
atgcccaaccgtctcggcatcgcctccatgtcccttggacgcccaggcatccactccctcccctggaagctccacgaagccgcccgccacggctacagcgggatcgagctcttcttcgacgacctggaccactacgcaaccacccacttcaatggcagccacatcgcggctgctcacgccgtgcacgctctctgcacgaccctcaacctcaccatcatctgcctgcaacccttctccttctacgaggggctcgtcgaccgcaagcaaaccgagtatctattgaccgtgaagctgcccacatggttccagctcgctcgcatcctcgacaccgacatgatccaggtgccctcgaacttcgcgcccgcccagcaaaccacgggtgaccgggacgtgatcgtcggcgacctccagcgcctcgcagacatcggcctggcacagtccccgcccttccgcttcgtatacgaagcactggcctggggcacgcgggtgaacctgtgggacgaggcgtacgagatcgtcgaggccgtggaccgtcccaacttcggtatctgtcttgatacgtttaaccttgcgggtcgggtgtatgcgcaccctggtcggcaggacgggaagacggtcaacgcggaggcggatctggctgcgtcgttgaagaagttgcgcgagacggtggatgtcaagaaggtgttctacgtgcaggttgtggatggagagaggctggagaggccgttggatgagacccatccgtttcatgtggaggggcagccggtgcggatgaactggagtcgcaatgcgaggttgtttgcgtttgaggaggatcgcggcgggtatttgcccattgaggagaccgcgagggcgttctttgatacggggttcgagggctgggtgtcgttggagttgtttagtcgcacgttggcggagaagggcacgggggtggtcacggagcatgcgagacgcgggttggagtcgtggaaggagttgtgtaggaggttggagtttaagggggcggagccgggactggattttgttcctggggaggtgaaggtgcagtcggttgctgtggggagtgggaagggggtggaacaggaggagatgggggttgtgcagcatcggttgtag

SEQ ID NO: 146 - DNA, 834 bp, Mycobacterium smegmatis
atgagtgccgagaggcgactgtcgctgaacaccatgaccaccaagcgcctcacgctgcgcgaggccgtcgaggcaaccgccgcggccgggctggagtccatcggcctgtggcgtgaccgcgtagccgaagcgggtgtggacaccgccgcgaaactgatgcacgacaacggtcttcgcgtgtccagtctgtgccggggcggtttcctgaccgggttcgaggaagaccatgcgctcgccgacaaccggcgcgccatcgaggaggcggtcacgctcgggacgcgagagctcgtcatggtcgtgggcggcatcccggaccgtgacctcgccgccgcgaggggacgtgtggctcagcggctcgagacgctcgtgccctacgccgtcgaccacggtgtccggctggcgctggaaccgctgcacccggtgttctgcgccgaccgcgcggtgatctccacactggggcaggcgctggcactcgcggcgccgtacccggccgaggccgtcggcgtcgtcgtcgacaccttccacgtgtggtgggatcccgagttggcggacggcatcgccgcggcgggcgctcagcaccggatcagctcgtaccaggtgtgcgactggctggtcccgatggccgccgacccgctggtgtcgcgcggcatgatgggtgacggcgtcatcgacttcggtgcggtcaccgcgatggtgcgggccgcgggatacgacggcgacgtcgaggtcgagatcttcaacgaggacatctgggccaccgacgcggccgtcgtcatcgacaccatgaaacagcgctaccgcgatctggtggcgcctgctctcacggcaggctga

SEQ ID NO: 147 - DNA, 1875 bp, Corynebacterium halotolerans
atgcgtacctcgatcgccaccgtctgcttgtccggcaccctcgcggagaagctccgggcggcggccgacgccggattcgacggcgtggagatcttcgagcaggatctcaccgtctccccgcactctccggagcagatccggcggcgcgccgccgacctgggcctcaccctcgatctcttccagcccttccgtgacttcgagggggtggaggaagcgcagttcgaggcgaacctgcgccgcatggaggcgaagttcgcgttgatgaaccgcctgggcatcgacaccatcctgctgtgctcgaacgtcgccaccgccaccatcgacgacgacgggctcttcgccgcccagctgcgccgcgccggtgaactggccgagcgttacgacgtgcgcatcgcctatgaggcgctggcctggggccgcttcgtcaacgacttcgagcacgcccgacgcatcgtcgacctggccggccacccgcgggtgggcacctgcctggacaccttccacatcctctcccgcggctggtccaccgacgcggtggaggagatcgcgggcgagaagatcttcttcgtccagctcgccgacgccccgcagctgagcatggacatcctgtcctggtcgcgccaccaccgcgtcttccccggcgagggggacttcgacctggtgaagttcatgcgccacctcgcgcgcaccggctacgacggtccggtctcgctggagatcttcaacgactccttccgcaaggccgaggtcggacgcaccgccgtcgacggcctgcgttccctgcggtggctggaggaccagacctggcgcgccctgcacgccgcgggggagggcaaggccgctgaagccctggagctgtccccgctgcccgaggtcgccgaccccgagggcgtggacttcgtggagatctccaccggccgactgggggagaccatcaaggtgctccaccagctcggcttccgcctcggcgggtaccaccgcagcaagccccagttccaggtgtggacccaggggccggtgcgcgtcgtcatcggcgaccgcgggccgaccggggcccccaccggcatcacctccctgggcgtgcggaccccggacccggccgccgcgcaggcccgtgcccacctgctccaggcccgtccggtcccccgcgaacgggccgcgggcgaggtcgagctgcacggggtgtacgcacccgacggcaccgaagtgttcttcagcggtctggcccccgagaccgccccggcgtggctggcggaattcggcgtcacggacaacgacctggagcccgccccgctgatcaccggcatcgaccacgtcaatctggcccagccctggcagcactatgacgagaccgtgctgttctacacctccctcatggcgctggagacccacagccgcgaggagttccccagccccatcgggctgatcagcaataaggtcatgcgttcggccaacgacaccgtgcggttactgctcagcgtcgcccccgaggacggtgagcagggtgacttcctggccgccgcctacccggagcacatcgccatcaccaccaccgacatcgtcgcagtggcgcgtcgtgcgcgacagcggggactggcgttcctgccggtccccgagaactactacgacgacctgcaggcgagattcgacctgaccccggccttcctcgccgaactgcgcgagaacgacctgctctacgaccgcgacgccgacggcgaattcctgcacttctacaccggcaccctgggcacgatgttcatcgaggtcgtcgagcgccgcggcggtttctccggctggggcgagaacaacgccccggtccgactcgccgcccagtaccgcaacgtgcgcgacgccgaacgcggcattccgcagtag

SEQ ID NO: 148 - DNA, 1935 bp, Rhodococcus opacus
atgggacgacaggttcgtacgagcgttgccacggtatccctgagcggatcgctggaggagaaggttaccgcgatcgcggcggccgggttcgacggattcgaggtgttcgaacccgatttcgtgagctcgccgtggtcgccgcgtgagctggcttcccgcgcagcggatctcggactcacactcgatctgtatcagccgttccgcgatctggactccgtggacgacacgacgttcgcgcgcaacctgatccgagccgagcgcaagttcgacatcatggagcagctcggctgcgacaccctgctggtgtgctcgtcgccgttgcccgaggcggtgcgggacgacgctcgcctgaccgagcaactccacactctcgccgagcgcgcacacagccggggtctccgcatcgcctacgaggcgctggcctggggcacgcacgtcaacacgtaccggcacgcgtggaagatcgtgcaggacgcggaccatcctgccctcggtacctgcctcgacagcttccacatcctctcccgcggcgacgacccgtccggcatccgcgacatcccgggggagaagatcttcttcctccaactcgccgacgcgccccgcatgtcgatggacatcctgcagtggagccggcaccaccggaacttcccggggcagggcaacttcgatctcgcgacgttcggcgcgcacgtccaggccgctggatacaccggaccgtggtcgctcgagatcttcaacgacacgttccggcagtcgtccacggggcgcacggccgccgacgcgcaccgctcgctgctgtacctccaggaggaggtcgcacgcgtgcaggccgagcgcggtgaggacaccggtcgcggcctgacgctgttcgagccgccgccgcgcgcacccctcgaaggcatcgtgtcgctccggctcgcggccggtccgggcaaggattccgaccttcggcaggcgctgcagcacatcggattccgtctggtgggccggcaccgcagccacgacctccagttgtggcggcacggccggatgaccatcgtggtcgatgcgaccgcgggcacggtgtggaccgctccgggtctgcctgcgcacctgccggtgctcacccagatcggtatccggtcgagcgatcccgacgcgtggggtgagcgcgccgcggcgctcgaggtcccggtgcacgaggtcctgttgcccggtgtcgacaccgcacccgaatcggatgtggtgcgtctcaagatcaccgacgcgacgtcgctggatctgcgcggcccgggcagcgccgcgtcgtggcagtcggcgttcgatctgtatccgacggagtcgcgctggcaggatgaggtgcccgtcttcaccggtgtcgatcacgtggcgctcgccgtgccgtccgacaactgggacggcatcatgctgctgctccgttcggtgttcgcgatggcgccgcacgagggcctcgatgtcaccgacgcggtcggaatgatgcgcagtcaggcgctgacgatggatcagacgggtgcggacggcgtcgaccgtccgctgcgcatctccctgaacatggttccgggtgcggtgtcgggcaactcccacatcgccgcggctcggcgcggcggcatcagtcacgtcgcgttctcgtgcacggacattttcaccgccgccgcgaccatgcagtccaacgggttcgagccccttgtgatttcgccgaactactacgacgacctcgaggcccgcttcgggctctcccgcgaactcctggaccggatgagcgggtcgggcatcatgtacgaccgtgatgcgcacggcgagttcttccatctgttcacccagacggtgggcgccgacctgttcttcgaggtggtgcaacgcgtcggcggttacgagggatacggggacgcgaactccgcgatgcgtttggcggcccagttgcgggcggctggctga

SEQ ID NO: 149 - DNA, 1101 bp, Aspergillus oryzae
atgcctaaccgtctcggaattggttccatgtccctggggcgcccgggaatccacgatctgccaaccaagctgcaccaggcctctcagttcggctacaagggcatcgagctattctttgacgaccttgaccacttggccaagttgctctttgatggagatcatattttagctgctcatcatgtacgccagctttgtgtttcgctgggcctctctatcatctgtctgcagcccttttggcactacgaggggcttctggatcgcactgagcacgagcgtcttctcactgaaaagcttcccaagtggtttgagcttgcacgcattctggatacagatctcatccagatcccatctaactttctccccgccgatgctcagacaggccagccccgcaccacaggtgacatgtctgtcattgtctcagatcttcagaagatcgccgatcttggccttcagcagtctcccccctttcgttttgtctacgaagccctagcatggggtaaccacatcaacaaatgggaagactcctgggaagttgtagagcgggtcaaccgtccaaactttggaatttgtcttgacaccttcaatatcgctggacgggtgtatgccgatcccacatctcccacaggaaagacgcctaatgcggaagccgacctccaggcatctatcgcccgcctgcgaactcgcatcgacctctcaaaggttttctatgttcaaatcgtggatggcgaacgcctgagtacccctctggacgaatctcacccattctatgtcaagggtcagccctcccgcatgaactggtcgcgtaacgcacgcctgtttgcctttgaagaggaccgtggtggatacttacccgtcttggacgtcgctaaagccttcttcgatattggcttcgagggctgggtttccctggaattgttcaacagaagcttggctgatcctgacccatctacgcctcgcaatcatgccaaaagagggtttgagtcttggaagaaactggtcgctgccttgaagctcaataccggtgatgcttctatggtgcatggtcttgacggtacaatttcaccatcgacttctgctttgcctgtgcagcatcgcctttag

SEQ ID NO: 150 - DNA, 843 bp, Bacillus thuringiensis
atgaaatattcgctatgtaccatttcatttcgtcatcaattaatttcatttactgatattgttcaatttgcatatgaaaacggttttgaaggaattgaattgtgggggactcatgcacaaaatttgtatatacaagaacgcgaaacgacagaacgagaattgacttttctaaaggataaaaacttagaaattacgatgataagtgattacttagatatatcattatcagcagattttgaaaaaacgatagagaaaagtgaacaacttgtagtactagctaattggtttaatacgaataaaattcgcacgtttgctgggcaaaaagggagcaaggacttctcggaacaagagagaaaagagtatgtaaagcgaatacgtaagatttgtgatgtgtttgctcagcacaatatgtatgtgctgttagaaacacatcccaatacactaacagacacattgccttctactatagaactattagaagaagtaaatcatccgaatttaaaaataaatcttgattttctccatatatgggagtctggcgcagatccaatagacagtttccatcgattaaagccgtggacactacattaccattttaagaatatatcttcagcggattatttgcatgtgtttgaacctaataatgtatatgctgcagcaggaagtcgtattggtatggttccgttatttgaaggtattgtaaattatgatgagattattcaggaagtgagaggtacggatctttttgcttccttagaatggtttggacataatgcaaaagagatattaaaagaagaaatgaaagtattaataaatagaaaattagaagtagtaacttcgtaa

SEQ ID NO: 151 - DNA, 2094 bp, Corynebacterium glutamicum
ttgacgctgtcacctgaacttcaggcgctcactgtacgcaattacccctctgattggtccgatgtggacaccaaggctgtagacactgttcgtgtcctcgctgcagacgctgtagaaaactgtggctccggccacccaggcaccgcaatgagcctggctccccttgcatacaccttgtaccagcgggttatgaacgtagatccacaggacaccaactgggcaggccgtgaccgcttcgttctttcttgtggccactcctctttgacccagtacatccagctttacttgggtggattcggccttgagatggatgacctgaaggctctgcgcacctgggattccttgaccccaggacaccctgagtaccgccacaccaagggcgttgagatcaccactggccctcttggccagggtcttgcatctgcagttggtatggccatggctgctcgtcgtgagcgtggcctattcgacccaaccgctgctgagggcgaatccccattcgaccaccacatctacgtcattgcttctgatggtgacctgcaggaaggtgtcacctctgaggcatcctccatcgctggcacccagcagctgggcaacatcatcgtgttctgggatgacaaccgcatctccatcgaagacaacactgagatcgctttcaacgaggacgttgttgctcgttacaaggcttacggctggcagaccattgaggttgaggctggcgaggacgttgcagcaatcgaagctgcagtggctgaggctaagaaggacaccaagcgacctaccttcatccgcgttcgcaccatcatcggcttcccagctccaaccatgatgaacaccggtgctgtgcacggtgctgctcttggcgcagctgaggttgcagcaaccaagactgagcttggattcgatcctgaggctcacttcgcgatcgacgacgaggtcatcgctcacacccgctccctcgcagagcgcgctgcagagaagaaggctgcatggcaggtcaagttcgatgagtgggcagctgccaaccctgagaacaaggctctgttcgatcgcctgaactcccgtgagcttccagcgggctacgctgacgagctcccaacatgggatgcagatgagaagggcgtcgcaactcgtaaggcgtccgaggctgcacttcaggcactgggcaagacccttcctgagctgtggggcggttccgctgacctcgcaggttccaacaacaccgtgatcaagggctccccttccttcggccctgagtccatctccaccgagacctggtctgctgagccttacggccgtaacctgcacttcggtatccgtgagcacgctatgggatccatcctcaacggcatttccctccacggtggcacccgcccatacggcggaaccttcctcatcttctccgactacatgcgtcctgcagttcgtcttgcagctctcatggagaccgacgcttactacgtctggacccacgactccatcggtctgggcgaagatggcccaacccaccagcctgttgaaaccttggctgcactgcgcgccatcccaggtctgtccgtcctgcgtcctgcagatgcgaatgagaccgcccaggcttgggctgcagcacttgagtacaatgaaggccctaagggtcttgcactgacccgccagaacgttcctgttctggaaggcaccaaggagaaggctgctgaaggcgttcgccgcggtggctacgtcctggttgagggttccaaggaaaccccagatgtgatcctcatgggctccggctccgaggttcagcttgcagttaacgctgcgaaggctctggaagctgagggcgttgcagctcgcgttgtttccgttccttgcatggattggttccaggagcaggacgcagagtacatcgagtccgttctgcctgcagctgtgaccgctcgtgtgtctgttgaagctggcatcgcaatgccttggtaccgcttcttgggcacccagggccgtgctgtctcccttgagcacttcggtgcttctgcggattaccagaccctgtttgagaagttcggcatcaccaccgatgcagtcgtggcagcggccaaggactccattaacggttaa

SEQ ID NO: 152 - DNA, 1083 bp, Corynebacterium glutamicum
atgtctcacattgatgatctggcacagctcggcacttccacttggctcgacgacctctcccgcgagcgcattacttccggcaatctcagccaggttattgaggaaaagtctgtagtcggtgtcaccaccaacccagctattttcgcagcagcaatgtccaagggcgattcctacgacgctcagatcgcagagctcaaggccgctggcgcatctgttgaccaggctgtttacgccatgagcatcgacgacgttcgcaatgcttgtgatctgtttaccggcatcttcgagtcctccaacggctacgacggccgcgtgtccatcgaggttgacccacgtatctctgcggaccgcgacgcaaccctggctcaggccaaggagctgtgggcaaaggttgatcgtccaaacgtcatgatcaagatccctgctaccccaggttctttgccagcaatcaccgacgctttggctgagggcatcagtgttaacgtcaccttgatcttctccgttgctcgctaccgcgaagtcatcgctgcgttcatcgagggcatcaagcaggcagctgcaaacggccacgacgtatccaagatccactctgtggcttccttcttcgtctcccgcgtcgacgttgagatcgacaagcgcctcgaggcaatcggatccgatgaggctttggctctgcgtggcaaggcaggcgttgccaacgctcagcgcgcttacgctgtgtacaaggagcttttcgacgccgccgagctgcctgaaggcgccaacactcagcgcccactgtgggcatccaccggcgtgaagaaccctgcgtacgctgcaactctttacgtttccgagctggctggtccaaacaccgtcaacaccatgccagaaggcaccatcgacgctgttctggaactgggcaacctgcacggtgacaccctgtccaactccgcggcagaagctgacgctgtgttctcccagcttgaggctctgggcgttgacttggcagatgtcttccaggtcctggagaccgagggcgtggacaagttcgttgcttcttggagcgaactgcttgagtccatggaagctcgcctgaagtag

SEQ ID NO: 153 - DNA, 1098 bp, Corynebacterium glutamicum
atgagcgcagcgcagattttcaacaccgtccacgtcaatggatcttccccctatgatgtccacattggttccggcctcaacgagctcattgttcagcgcgcagcggaatcaggcgcggagcaggtagcgattttgcaccagcccagcatggatgacattgcatccgagttggatgcagcactagtcgctgctggtttgaaggtcctgcaccttaatgttcccgatgcggaaaacggcaagtccttggaagtagcggggcagtgctgggatgaattgggtggcgcagcattcggccgccgcgatatcgtcatcggacttggtggcggtgctgccacagatctcgcgggattcgtcgctgctgcgtggatgcgtggcgtgcgcgtcattcaggttccaaccaccttgttggccatggtggacgctgcggtgggcggcaagactggcatcaataccgccgcaggcaagaaccttgtgggcgcgttccacgagcctgacgcagtattcattgacaccgaacgcctagccaccctgcctgacgcggaaatcatcgcgggatccgccgaaatcatcaaaactggtttcatcgccgacccagaaatcctgcgcctttacgaaactgatcccgcagcctgcctgaagaaagaagtcgaaggctcccacctacctgaactgatttggcgctccgtcaccgtcaagggctccgtggtcggccaagacctcaaagaatctagcctgcgcgaaatcctcaactacggacacacctttgcccacgccgtcgaactccgcgaaaacttccgctggcgccacggcaatgccgttgcagtgggcatgatgttcatcgctaacctctcccacaagctcgggcttatcgacgcgcccctcctcgagcgccaccgctcaatcctggcggccatcggtctgcccacttcctacgaaggcggagccttcgacgagctttacgacggcatgacccgcgacaagaaaaaccgcgacggcaacatccgcttcgtcgcactgaccgccgtgggcgaggttacccgcattgaggggccctcaaaacaagatttacagagtgcttatgaggcaatcagccactaa

SEQ ID NO: 154 - DNA, 573 bp, Corynebacterium glutamicum
atggagcgtaatgaagtgaatgatcaaattcacttagatcatcaatcagatgacacctctgaatgctcctgcccgatcgtggttcttgtgggtttgccaggagctggaaaatccaccattggacgtcgattagcgcgcgccttaaacactgaactcgtcgactccgacgaactcattgagcgcgccaccggaaaagcctgcggcgccgtgttcagcgagctcggcgagccagccttccgcgagctcgaggccatccacgtggccgaagcactgaaatcctccggagtggtgagcttgggaggcggatctgtgctgacagaatccacccgtgaactgctcaaaggccacgacgtggtctggatcgacgtgccagtagaagaaggcatcaggcgcaccgcaaacgagcgttcccgccccgtgctgcaagccgccgaccccgccgagcactaccgcaacctggtgaaagtgcgcaccccgttgtacgaagaggtggcaacctaccgacttcgcaccaacaaccgcagcccccagcaagtggtggcagcagtgttgcatcatctagaaatcgattaa

SEQ ID NO: 155 - DNA, 1293 bp, Corynebacterium glutamicum; identical to SEQ ID NO: 4

SEQ ID NO: 156 - DNA, 1233 bp, Corynebacterium glutamicum
atgctaggcatgcttcgatggactacagcaggtgaatcccacggccaggcgcttatcgccacggttgaacacatgccagcaggcgtgcccgtgactaaagatgaggtctcgtatcaattggcgcgccgacgccttggatatggtcgcggcgctcgcatgaagtttgagcaagacgcgttgaccttcctgaccggcatccgccacggcctcactttgggtagccccatctcaatcatgatcggcaacactgagtgggataagtggaccaccatcatgtcctctgacgctttggacatggaagacccagacaacgttgcggcgatgtcttcgggtcgcggtgcaaaactgactcgtccgcgtccaggccacgcagattacgcaggcatgctcaagtacggattcgatgatgcccgcaacgtgctggagcgttcttcagcccgtgagacggcagctcgcgtggcagcagcaaccgttgcgcgttccttcctccgtgaaaccttgggcgtggaggtgctctctcacgtaatttccattggtgcgtccgagccttacgtcggcgcggagccaacctttgcagatattcaagcaatcgatgattccccagttcgtgcattcggtaaagacgctgaaaaatccatgatcgcggaaatcgaggccgcaaagaaagccggcgataccctcggtggcatcgtggaagtgattgttgaaggcctacccatcggtttgggctcacacatttctggcgaagatcgcctcgatgcgcagatcgcagctgcactcatgggcattcaggccatcaagggcgtggaaatcggtgacggtttcgaagaagctcgtcgacgtggctccgaagcccacgatgaagtgttcctggatgacaacggcgtataccgcaacaccaaccgtgcaggtggcctcgaaggcggcatgaccaacggtgaaaccctgcgcgttcgtgctggcatgaagccaatttctactgtgcctcgcgccctgaaaaccattgatatggaaaacggcaaggcagcaaccggaatccaccagcgttccgacgtgtgcgctgttccagccgccggtgtcgttgcagaagcaatggtcaccctggttctcgcccgcgcagtcctgcagaaattcggcggtgactccctgagtgaaaccaagagcaacattgacacctacctcaaaaacattgaggaacgaatgaaattcgaaggtttagaggatggagcgtaa

SEQ ID NO: 157 - DNA, 1476 bp, Corynebacterium glutamicum
atggctagtaccttcattcaggccgacagccctgaaaaaagtaagaagctacccccactcacagaaggtccgtatagaaagcggctgttctacgttgcactagttgcgacgtttggtgggctgctcttcggatatgacaccggagtaatcaacggtgcactcaacccaatgacacgtgagctcggactaaccgcgttcaccgagggtgttgtaacttcttccctgctgtttggtgcagcagctggtgcgatgtttttcggtcgcatttccgacaactggggtcgccggaaaacaatcatctcacttgcagtagctttctttgtcggcaccatgatctgcgtgtttgctccatcttttgcagtaatggttgtcggacgtgtgcttcttggactcgcagttggtggcgcttccactgttgtccctgtctacctggctgaacttgctccttttgaaatccgtggctcactggctggccgtaatgagttgatgattgttgttggtcagctcgcagctttcgtcatcaatgcgattattggaaatgtttttggacaccacgatggtgtgtggcgctacatgctggcaattgccgcaatcccagcaattgccctcttctttggaatgctccgagttccagaatccccacgctggcttgttgagcgaggacgcattgatgaggctcgcgcagttcttgaaaccattcgccctctagaacgtgcccatgcagaagttgctgatgttgagcacctagcaaaagaagagcacgccatttccgagaagtccatgggcttaagggaaattttgtccagcaagtggcttgtgcgcatcctcctggtaggtatcggattgggtgtcgcacagcagctgactggcatcaactccatcatgtactacggccaggttgttctcattgaggctggtttctccgaaaatgcagctctgatcgccaacgtggcgccaggagtgatcgcagttgtcggtgcatttatcgcactgtggatgatggatcgcatcaaccgccgtaccaccctcattaccggctactctctcactaccattagccacgtgttgatcggcatcgcatccgtagcattctcagtcggcgatccacttcgcccatacgttattttgaccctagttgtgatcttcgtaggatccatgcagaccttcctcaacgtagccacctgggtcatgctctccgagctcttcccgctggcaatgcgaggtttcgcaatcggtatctcagtgttcttcctctggatcgcaaacgcgttcctcggattgttcttccccaccatcatggaagcagtaggactaaccggaaccttcttcatgttcgccggaatcggtgtggttgccttgatcttcatctacacccaggttcctgaaactcgtggacgtaccttggaggagattgatgaggatgttacttccggtgtcattttcaacaaggacatccgaaaaggaaaggtgcactaa

SEQ ID NO: 158 - DNA, 972 bp, Corynebacterium glutamicum
atgccacaaaaaccggccagtttcgcggtgggctttgacatcggcggcaccaacatgcgagctgggcttgtcgacgaatccgggcgcatcgtgaccagtttgtcggcgccgtcgccgcgcacgacgcaggcaatggaacaggggatttttgatctagtcgaacagctcaaggccgaatacccggttggtgctgtgggacttgccgtcgcgggatttttggatcctgagtgcgaggttgttcgatttgccccgcaccttccttggcgcgatgagccagtgcgtgaaaagttggaaaaccttttgggcctgcctgttcgtttggaacatgatgccaactcagcagcgtggggtgagcatcgttttggtgcagctcaaggcgctgacaactgggttttgttggcactcggcactggaattggtgcagcgctgattgaaaaaggcgaaatttaccgtggtgcatatggcacggcaccagaatttggtcatttgcgtgttgttcgtggcggacgcgcatgtgcgtgtggcaaagaaggctgcctggagcgttactgttccggtactgccttggtttacactgcgcgtgaattggcttcgcatggctcattccgcaacagcgggctgtttgacaagatcaaagccgatccgaattccatcaatggaaaaacgatcactgcggcagcgcgccaagaagacccacttgctctcgccgttctggaagatttcagcgagtggctgggcgaaactttggcgatcattgctgatgtccttgacccaggtatgatcatcattggtggcggactgtccaatgctgccgacctttatttggatcgctcggttaaccactattccacccgcatcgtcggcgcaggatatcgccctttggcacgcgttgccacagctcagttgggtgcggatgctggcatgatcggtgtcgctgatctggctcgacgttccgtgttggaagccaactag

SEQ ID NO: 159 - DNA, 912 bp, Corynebacterium glutamicum
atgactgatcccacttgcacccttgcccttgatattggtgccacaaagattgcctacgcactagtccccgataacgccccgacgacaacattgtccacgggacgcttgggaacaaaagaaggcgacagccctatcgagcagatccggctggttcttctggcaggcttaaaagctgccgaggaacacggtctcagtgtcgcccgcatcggcatgggcgctcctggtgtaattctgggaccagagggaaccatcgtgtacaacggtgaaaccctcacagagtgggcaggcactgacctgcgaggattatcccgagaagtcctcaacgttccattcgcggcacacaatgatgtccgcgtatgggcctacggtgagcaccacttaggcaccggcaaagacctcaccggcagggttctctacgtgtccctcggcactggagtcggcggagcaatcatcgaagacggaatcatgatgagtagccccactggaactgcgggagaattcgcagaagttgtgtgctctgaccatgcaggattagccgttcggtgcgaaaatgtagcaagtggcaccggcctaaccaggtactacaacgaggccgccgcaactcaacttgaccttcccgccatcatggagcgcttccaccaaggtgacggcctggcacagcaaatcattactggaaatctccgaggctttggccaagcgctaggcgcattagtcacagtgctggacctttccgcagtagtagttggaggcggagtcgcaggcatcggcgcacccgtcatggatcccatcaccgcagggattttcgatcgaatgttagcccccaacaaatccgtacaagttttaagcacgtcccttggtgcccaagcagccgtcatcgcagcagcaaaatatgcccgcgataacgccttttaa

SEQ ID NO: 160 - DNA, 1233 bp, Corynebacterium glutamicum
gtggcgcgcggcggtgtacagcaccccggtgaccacattgatcacagcacctgctacgacctcgccgtcgatcgccgcagcgatcgagacggcgtattggggcaggccataaaggaagttgacggtgccgtcaatggggtcgacgatccaggtaactccgcttatcgacgccgtccccgtcccttcctcgcctatcagcccgtctttaggccgaagttcctgcaacctattggcgataaaatcttcagccaaagtatctactatcgtcaccggatcgactgtcgaacttttggtgttggtgtagtcccacaaattggtgagttcagcacgtttatccctgatacgtgtagcggtaagcgtggcagtttccgcggcgatggcacgcaactcattaaacgattgttgttccataagaccatcatcgttgtttttttagaaaattgcctgccaaaagccgaagtaatttgtacacttgggcgcatgactgagactggatttggaattgatatcggtggctccggcatcaaaggcgcccgcgttaaccttaagaccggtgagtttattgatgaacgcataaaaatcgccacccctaagccagcaaccccagaggctgtcgccgaagtagtcgcagagattatttctcaagccgaatgggagggtccggtcggaattaccctgccgtctgtcgttcgcgggcagatcgcgctatccgcagccaacattgacaagtcctggatcggcaccgatgtgcacgaactttttgaccgccacctaaatggccgagagatcaccgttctcaatgacgcagacgccgccggcatcgccgaagcaacctttggcaacgctgccgcacgcgaaggcgcagtcatcctgctgacccttggtacaggtattggatccgcattccttgtggatggccaactgttccccaacacagaactcggtcacatgatcgttgacggcgaggaagcagaacaccttgcagcagcagccgtcaaagaaaacgaagatctgtcatggaagaaatgggcgaagcgcctgaacaaggtgctgagcgaatacgagaaacttttctccccatccgtcttcatcatcggtggcggaatttccagaaagcacgaaaagtggcttccattgctggagctagacactgacattgtcccagctgagctgcgcaatcgagccggaatcgtaggagctgccatggcagtaaaccaacacctcaccccataa

SEQ ID NO: 161 - DNA, 1005 bp, Corynebacterium glutamicum
atgaccattcgtgttggtattaacggatttggccgtatcggacgtaacttcttccgcgcagttctggagcgcagcgacgatctcgaggtagttgcagtcaacgacctcaccgacaacaagaccctttccacccttctcaagttcgactccatcatgggccgccttggccaggaagttgaatacgacgatgactccatcaccgttggtggcaagcgcatcgctgtttacgcagagcgcgatccaaagaacctggactgggctgcacacaacgttgacatcgtgatcgagtccaccggcttcttcaccgatgcaaacgcggctaaggctcacatcgaagcaggtgccaagaaggtcatcatctccgcaccagcaagcaacgaagacgcaaccttcgtttacggtgtgaaccacgagtcctacgatcctgagaaccacaacgtgatctccggcgcatcttgcaccaccaactgcctcgcaccaatggcaaaggtcctgaacgacaagttcggcatcgagaacggcctcatgaccaccgttcacgcatacaccggcgaccagcgcctgcacgatgcacctcacggcgacctgcgtcgtgcacgtgcagcagcagtcaacatcgttcctacctccaccggtgcagctaaggctgttgctctggttctcccagagctcaagggcaagcttgacggctacgcacttcgcgttccagttatcaccggttccgcaaccgacctgaccttcaacaccaagtctgaggtcaccgttgagtccatcaacgctgcaatcaaggaagctgcagtcggcgagttcggcgagaccctggcttactccgaagagccactggtttccaccgacatcgtccacgattcccacggctccatcttcgacgctggcctgaccaaggtctccggcaacaccgtcaaggttgtttcctggtacgacaacgagtggggctacacctgccagctcctgcgtctgaccgagctcgtagcttccaagctctaa

SEQ ID NO: 162 - DNA, 1053 bp, Escherichia coli
atgaattatcagaacgacgatttacgcatcaaagaaatcaaagagttacttcctcctgtcgcattgctggaaaaattccccgctactgaaaatgccgcgaatacggttgcccatgcccgaaaagcgatccataagatcctgaaaggtaatgatgatcgcctgttggttgtgattggcccatgctcaattcatgatcctgtcgcggcaaaagagtatgccactcgcttgctggcgctgcgtgaagagctgaaagatgagctggaaatcgtaatgcgcgtctattttgaaaagccgcgtaccacggtgggctggaaagggctgattaacgatccgcatatggataatagcttccagatcaacgacggtctgcgtatagcccgtaaattgctgcttgatattaacgacagcggtctgccagcggcaggtgagtttctcgatatgatcaccccacaatatctcgctgacctgatgagctggggcgcaattggcgcacgtaccaccgaatcgcaggtgcaccgcgaactggcatcagggctttcttgtccggtcggcttcaaaaatggcaccgacggtacgattaaagtggctatcgatgccattaatgccgccggtgcgccgcactgcttcctgtccgtaacgaaatgggggcattcggcgattgtgaataccagcggtaacggcgattgccatatcattctgcgcggcggtaaagagcctaactacagcgcgaagcacgttgctgaagtgaaagaagggctgaacaaagcaggcctgccagcacaggtgatgatcgatttcagccatgctaactcgtccaaacaattcaaaaagcagatggatgtttgtgctgacgtttgccagcagattgccggtggcgaaaaggccattattggcgtgatggtggaaagccatctggtggaaggcaatcagagcctcgagagcggggagccgctggcctacggtaagagcatcaccgatgcctgcatcggctgggaagataccgatgctctgttacgtcaactggcgaatgcagtaaaagcgcgtcgcgggtaa